European Patent Specification EP 3 456 738 B1, published July 17, 2024. Title: Antibody variants. Applicant: Tillotts Pharma AG. The sequence listing filed with the application follows.

SEQUENCE LISTING (24 sequences)

SEQ ID NO: 1 - protein, 221 aa, Artificial Sequence
  Light chain of Ab-wt, the parent antibody of the modified antibodies used in the examples (clone 16-22-H05)
DIQMTQSPSSLSASVGDRVTIKCQASQSIFSGLAWYQQKPGKAPKLLIYGASKLASGVPSRFSGSGSGTEFTLTISGLQPADFATYYCQSYYYSSSSSDGSYAFGGGTKLTVLGRTVAAPSVFIFPPSDEQLKSGTASVVCLLNNFYPREAKVQWKVDNALQSGNSQESVTEQDSKDSTYSLSSTLTLSKADYEKHKVYACEVTHQGLSSPVTKSFNRGEC

SEQ ID NO: 2 - protein, 452 aa, Artificial Sequence
  Heavy chain of Ab-wt, the parent antibody of the modified antibodies used in the examples (clone 16-22-H05)
EVQLVESGGGLVQPGGSLRLSCKASGIDFNNYGIGWVRQAPGKGLEWITYIYPGFAITNFANSVKGRFTISSDNSKNTVYLQMNSLRAEDTAVYYCARDPVYATSSGYFDLWGQGTLVTVSSASTKGPSVFPLAPSSKSTSGGTAALGCLVKDYFPEPVTVSWNSGALTSGVHTFPAVLQSSGLYSLSSVVTVPSSSLGTQTYICNVNHKPSNTKVDKKVEPKSCDKTHTCPPCPAPELLGGPSVFLFPPKPKDTLMISRTPEVTCVVVDVSHEDPEVKFNWYVDGVEVHNAKTKPREEQYNSTYRVVSVLTVLHQDWLNGKEYKCKVSNKALPAPIEKTISKAKGQPREPQVYTLPPSREEMTKNQVSLTCLVKGFYPSDIAVEWESNGQPENNYKTTPPVLDSDGSFFLYSKLTVDKSRWQQGNVFSCSVMHEALHNHYTQKSLSLSPGK

SEQ ID NO: 3 - protein, 11 aa, Artificial Sequence
  CDR L1 of clone 16-22-H05
QASQSIFSGLA

SEQ ID NO: 4 - protein, 7 aa, Artificial Sequence
  CDR L2 of clone 16-22-H05
GASKLAS

SEQ ID NO: 5 - protein, 15 aa, Artificial Sequence
  CDR L3 of clone 16-22-H05
QSYYYSSSSSDGSYA

SEQ ID NO: 6 - protein, 10 aa, Artificial Sequence
  CDR H1 of clone 16-22-H05
GIDFNNYGIG

SEQ ID NO: 7 - protein, 17 aa, Artificial Sequence
  CDR H2 of clone 16-22-H05
YIYPGFAITNFANSVKG

SEQ ID NO: 8 - protein, 13 aa, Artificial Sequence
  CDR H3 of clone 16-22-H05
DPVYATSSGYFDL

SEQ ID NO: 9 - protein, 122 aa, Artificial Sequence
  VH of humanized IgG of clone 16-22-H05
EVQLVESGGGLVQPGGSLRLSCKASGIDFNNYGIGWVRQAPGKGLEWITYIYPGFAITNFANSVKGRFTISSDNSKNTVYLQMNSLRAEDTAVYYCARDPVYATSSGYFDLWGQGTLVTVSS

SEQ ID NO: 10 - protein, 114 aa, Artificial Sequence
  VL of humanized IgG of clone 16-22-H05
DIQMTQSPSSLSASVGDRVTIKCQASQSIFSGLAWYQQKPGKAPKLLIYGASKLASGVPSRFSGSGSGTEFTLTISGLQPADFATYYCQSYYYSSSSSDGSYAFGGGTKLTVLG

SEQ ID NO: 11 - protein, 452 aa, Artificial Sequence
  Heavy chain of Ab-REW (based on clone 16-22-H05)
EVQLVESGGGLVQPGGSLRLSCKASGIDFNNYGIGWVRQAPGKGLEWITYIYPGFAITNFANSVKGRFTISSDNSKNTVYLQMNSLRAEDTAVYYCARDPVYATSSGYFDLWGQGTLVTVSSASTKGPSVFPLAPSSKSTSGGTAALGCLVKDYFPEPVTVSWNSGALTSGVHTFPAVLQSSGLYSLSSVVTVPSSSLGTQTYICNVNHKPSNTKVDKKVEPKSCDKTHTCPPCPAPELLGGPSVFLFPPKPKDTLMISRTPEVTCVVVDVSHEDPEVKFNWYVDGVEVHNAKTKPREEQYNSTYRVVSVLTVLHRDWLNGKEYKCKVSNKALPAPIEKTISKAKGQPREPQVYTLPPSREEMTKNQVSLTCLVKGFYPSDIAVEWESNGQPENNYKTTPPVLDSDGSFFLYSKLTVDKSRWQQGNVFSCSVEHEALHWHYTQKSLSLSPGK

SEQ ID NO: 12 - protein, 454 aa, Artificial Sequence
  Heavy chain of Ab-REW (based on clone 17-22-B03)
EVQLVESGGGLVQPGGSLRLSCKASGIDFSAGYDMCWVRQAPGKGLEWIACIDSRREESDYASWAKGRFTISKDSSKNTVYLQMNSLRAEDTAVYYCARGGYGGDGVDGAFDPWGQGTLVTVSSASTKGPSVFPLAPSSKSTSGGTAALGCLVKDYFPEPVTVSWNSGALTSGVHTFPAVLQSSGLYSLSSVVTVPSSSLGTQTYICNVNHKPSNTKVDKKVEPKSCDKTHTCPPCPAPELLGGPSVFLFPPKPKDTLMISRTPEVTCVVVDVSHEDPEVKFNWYVDGVEVHNAKTKPREEQYNSTYRVVSVLTVLHRDWLNGKEYKCKVSNKALPAPIEKTISKAKGQPREPQVYTLPPSREEMTKNQVSLTCLVKGFYPSDIAVEWESNGQPENNYKTTPPVLDSDGSFFLYSKLTVDKSRWQQGNVFSCSVEHEALHWHYTQKSLSLSPGK

SEQ ID NO: 13 - protein, 232 aa, Artificial Sequence
  Fc region of Ab-REW (including hinge region)
EPKSCDKTHTCPPCPAPELLGGPSVFLFPPKPKDTLMISRTPEVTCVVVDVSHEDPEVKFNWYVDGVEVHNAKTKPREEQYNSTYRVVSVLTVLHRDWLNGKEYKCKVSNKALPAPIEKTISKAKGQPREPQVYTLPPSREEMTKNQVSLTCLVKGFYPSDIAVEWESNGQPENNYKTTPPVLDSDGSFFLYSKLTVDKSRWQQGNVFSCSVEHEALHWHYTQKSLSLSPGK

SEQ ID NO: 14 - protein, 11 aa, Artificial Sequence
  CDR L1 of clone 17-22-B03
QASQSISSYLA

SEQ ID NO: 15 - protein, 7 aa, Artificial Sequence
  CDR L2 of clone 17-22-B03
KASTLAS

SEQ ID NO: 16 - protein, 13 aa, Artificial Sequence
  CDR L3 of clone 17-22-B03
QCTYYEPSYVFRA

SEQ ID NO: 17 - protein, 11 aa, Artificial Sequence
  CDR H1 of clone 17-22-B03
GIDFSAGYDMC

SEQ ID NO: 18 - protein, 17 aa, Artificial Sequence
  CDR H2 of clone 17-22-B03
CIDSRREESDYASWAKG

SEQ ID NO: 19 - protein, 14 aa, Artificial Sequence
  CDR H3 of clone 17-22-B03
GGYGGDGVDGAFDP

SEQ ID NO: 20 - protein, 124 aa, Artificial Sequence
  VH of humanized IgG of clone 17-22-B03
EVQLVESGGGLVQPGGSLRLSCKASGIDFSAGYDMCWVRQAPGKGLEWIACIDSRREESDYASWAKGRFTISKDSSKNTVYLQMNSLRAEDTAVYYCARGGYGGDGVDGAFDPWGQGTLVTVSS

SEQ ID NO: 21 - protein, 112 aa, Artificial Sequence
  VL of humanized IgG of clone 17-22-B03 -(sc08)
DIQMTQSPSSLSASVGDRVTITCQASQSISSYLAWYQQKPGKAPKLLIYKASTLASGVPSRFSGSGSGTDFTLTISSLQPEDFATYYCQCTYYEPSYVFRAFGGGTKLTVLG

SEQ ID NO: 22 - protein, 112 aa, Artificial Sequence
  VL of humanized IgG of clone 17-22-B03 -(sc02)
DIQMTQSPSSLSASVGDRVTIKCQASQSISSYLAWYQQKPGKAPKLLIYKASTLASGVPSRFSGSGSGTEFTLTISDLEPADFATYYCQCTYYEPSYVFRAFGGGTKLTVLG

SEQ ID NO: 23 - protein, 219 aa, Artificial Sequence
  Light chain of humanized IgG of clone 17-22-B03 -(sc08)
DIQMTQSPSSLSASVGDRVTITCQASQSISSYLAWYQQKPGKAPKLLIYKASTLASGVPSRFSGSGSGTDFTLTISSLQPEDFATYYCQCTYYEPSYVFRAFGGGTKLTVLGRTVAAPSVFIFPPSDEQLKSGTASVVCLLNNFYPREAKVQWKVDNALQSGNSQESVTEQDSKDSTYSLSSTLTLSKADYEKHKVYACEVTHQGLSSPVTKSFNRGEC

SEQ ID NO: 24 - protein, 219 aa, Artificial Sequence
  Light chain of humanized IgG of clone 17-22-B03 -(sc02)
DIQMTQSPSSLSASVGDRVTIKCQASQSISSYLAWYQQKPGKAPKLLIYKASTLASGVPSRFSGSGSGTEFTLTISDLEPADFATYYCQCTYYEPSYVFRAFGGGTKLTVLGRTVAAPSVFIFPPSDEQLKSGTASVVCLLNNFYPREAKVQWKVDNALQSGNSQESVTEQDSKDSTYSLSSTLTLSKADYEKHKVYACEVTHQGLSSPVTKSFNRGEC